European Patent Application EP 4 516 906 A1, published March 5, 2025. Title: Mutant neurodegenerative disease-related proteins. Applicant: Tokyo Metropolitan Institute of Medical Science. The sequence listing filed with the application follows.

SEQUENCE LISTING (70 sequences)

SEQ ID NO: 1 - DNA, 420 bp, Homo sapiens
  source 1..420: mol_type = other DNA
  CDS 1..420
atggatgtattcatgaaaggactttcaaaggccaaggagggagttgtggctgctgctgagaaaaccaaacagggtgtggcagaagcagcaggaaagacaaaagagggtgttctctatgtaggctccaaaaccaaggagggagtggtgcatggtgtggcaacagtggctgagaagaccaaagagcaagtgacaaatgttggaggagcagtggtgacgggtgtgacagcagtagcccagaagacagtggagggagcagggagcattgcagcagccactggctttgtcaaaaaggaccagttgggcaagaatgaagaaggagccccacaggaaggaattctggaagatatgcctgtggatcctgacaatgaggcttatgaaatgccttctgaggaagggtatcaagactacgaacctgaagcc

SEQ ID NO: 2 - protein, 140 aa, Homo sapiens
MDVFMKGLSKAKEGVVAAAEKTKQGVAEAAGKTKEGVLYVGSKTKEGVVHGVATVAEKTKEQVTNVGGAVVTGVTAVAQKTVEGAGSIAAATGFVKKDQLGKNEEGAPQEGILEDMPVDPDNEAYEMPSEEGYQDYEPEA

SEQ ID NO: 3 - DNA, 1056 bp, Homo sapiens
  source 1..1056: mol_type = other DNA
  CDS 1..1056
atggctgagccccgccaggagttcgaagtgatggaagatcacgctgggacgtacgggttgggggacaggaaagatcaggggggctacaccatgcaccaagaccaagagggtgacacggacgctggcctgaaagctgaagaagcaggcattggagacacccccagcctggaagacgaagctgctggtcacgtgacccaagctcgcatggtcagtaaaagcaaagacgggactggaagcgatgacaaaaaagccaagggggctgatggtaaaacgaagatcgccacaccgcggggagcagcccctccaggccagaagggccaggccaacgccaccaggattccagcaaaaaccccgcccgctccaaagacaccacccagctctggtgaacctccaaaatcaggggatcgcagcggctacagcagccccggctccccaggcactcccggcagccgctcccgcaccccgtcccttccaaccccacccacccgggagcccaagaaggtggcagtggtccgtactccacccaagtcgccgtcttccgccaagagccgcctgcagacagcccccgtgcccatgccagacctgaagaatgtcaagtccaagatcggctccactgagaacctgaagcaccagccgggaggcgggaaggtgcaaatagtctacaaaccagttgacctgagcaaggtgacctccaagtgtggctcattaggcaacatccatcataaaccaggaggtggccaggtggaagtaaaatctgagaagcttgacttcaaggacagagtccagtcgaagattgggtccctggacaatatcacccacgtccctggcggaggaaataaaaagattgaaacccacaagctgaccttccgcgagaacgccaaagccaagacagaccacggggcggagatcgtgtacaagtcgccagtggtgtctggggacacgtctccacggcatctcagcaatgtctcctccaccggcagcatcgacatggtagactcgccccagctcgccacgctagctgacgaggtgtctgcctccctggccaagcagggtttg

SEQ ID NO: 4 - protein, 352 aa, Homo sapiens
MAEPRQEFEVMEDHAGTYGLGDRKDQGGYTMHQDQEGDTDAGLKAEEAGIGDTPSLEDEAAGHVTQARMVSKSKDGTGSDDKKAKGADGKTKIATPRGAAPPGQKGQANATRIPAKTPPAPKTPPSSGEPPKSGDRSGYSSPGSPGTPGSRSRTPSLPTPPTREPKKVAVVRTPPKSPSSAKSRLQTAPVPMPDLKNVKSKIGSTENLKHQPGGGKVQIVYKPVDLSKVTSKCGSLGNIHHKPGGGQVEVKSEKLDFKDRVQSKIGSLDNITHVPGGGNKKIETHKLTFRENAKAKTDHGAEIVYKSPVVSGDTSPRHLSNVSSTGSIDMVDSPQLATLADEVSASLAKQGL

SEQ ID NO: 5 - DNA, 1143 bp, Homo sapiens
  source 1..1143: mol_type = other DNA
  CDS 1..1143
atggctgagccccgccaggagttcgaagtgatggaagatcacgctgggacgtacgggttgggggacaggaaagatcaggggggctacaccatgcaccaagaccaagagggtgacacggacgctggcctgaaagaatctcccctgcagacccccactgaggacggatctgaggaaccgggctctgaaacctctgatgctaagagcactccaacagcggaagctgaagaagcaggcattggagacacccccagcctggaagacgaagctgctggtcacgtgacccaagctcgcatggtcagtaaaagcaaagacgggactggaagcgatgacaaaaaagccaagggggctgatggtaaaacgaagatcgccacaccgcggggagcagcccctccaggccagaagggccaggccaacgccaccaggattccagcaaaaaccccgcccgctccaaagacaccacccagctctggtgaacctccaaaatcaggggatcgcagcggctacagcagccccggctccccaggcactcccggcagccgctcccgcaccccgtcccttccaaccccacccacccgggagcccaagaaggtggcagtggtccgtactccacccaagtcgccgtcttccgccaagagccgcctgcagacagcccccgtgcccatgccagacctgaagaatgtcaagtccaagatcggctccactgagaacctgaagcaccagccgggaggcgggaaggtgcaaatagtctacaaaccagttgacctgagcaaggtgacctccaagtgtggctcattaggcaacatccatcataaaccaggaggtggccaggtggaagtaaaatctgagaagcttgacttcaaggacagagtccagtcgaagattgggtccctggacaatatcacccacgtccctggcggaggaaataaaaagattgaaacccacaagctgaccttccgcgagaacgccaaagccaagacagaccacggggcggagatcgtgtacaagtcgccagtggtgtctggggacacgtctccacggcatctcagcaatgtctcctccaccggcagcatcgacatggtagactcgccccagctcgccacgctagctgacgaggtgtctgcctccctggccaagcagggtttg

SEQ ID NO: 6 - protein, 381 aa, Homo sapiens
MAEPRQEFEVMEDHAGTYGLGDRKDQGGYTMHQDQEGDTDAGLKESPLQTPTEDGSEEPGSETSDAKSTPTAEAEEAGIGDTPSLEDEAAGHVTQARMVSKSKDGTGSDDKKAKGADGKTKIATPRGAAPPGQKGQANATRIPAKTPPAPKTPPSSGEPPKSGDRSGYSSPGSPGTPGSRSRTPSLPTPPTREPKKVAVVRTPPKSPSSAKSRLQTAPVPMPDLKNVKSKIGSTENLKHQPGGGKVQIVYKPVDLSKVTSKCGSLGNIHHKPGGGQVEVKSEKLDFKDRVQSKIGSLDNITHVPGGGNKKIETHKLTFRENAKAKTDHGAEIVYKSPVVSGDTSPRHLSNVSSTGSIDMVDSPQLATLADEVSASLAKQGL

SEQ ID NO: 7 - DNA, 1230 bp, Homo sapiens
  source 1..1230: mol_type = other DNA
  CDS 1..1230
atggctgagccccgccaggagttcgaagtgatggaagatcacgctgggacgtacgggttgggggacaggaaagatcaggggggctacaccatgcaccaagaccaagagggtgacacggacgctggcctgaaagaatctcccctgcagacccccactgaggacggatctgaggaaccgggctctgaaacctctgatgctaagagcactccaacagcggaagatgtgacagcacccttagtggatgagggagctcccggcaagcaggctgccgcgcagccccacacggagatcccagaaggaaccacagctgaagaagcaggcattggagacacccccagcctggaagacgaagctgctggtcacgtgacccaagctcgcatggtcagtaaaagcaaagacgggactggaagcgatgacaaaaaagccaagggggctgatggtaaaacgaagatcgccacaccgcggggagcagcccctccaggccagaagggccaggccaacgccaccaggattccagcaaaaaccccgcccgctccaaagacaccacccagctctggtgaacctccaaaatcaggggatcgcagcggctacagcagccccggctccccaggcactcccggcagccgctcccgcaccccgtcccttccaaccccacccacccgggagcccaagaaggtggcagtggtccgtactccacccaagtcgccgtcttccgccaagagccgcctgcagacagcccccgtgcccatgccagacctgaagaatgtcaagtccaagatcggctccactgagaacctgaagcaccagccgggaggcgggaaggtgcaaatagtctacaaaccagttgacctgagcaaggtgacctccaagtgtggctcattaggcaacatccatcataaaccaggaggtggccaggtggaagtaaaatctgagaagcttgacttcaaggacagagtccagtcgaagattgggtccctggacaatatcacccacgtccctggcggaggaaataaaaagattgaaacccacaagctgaccttccgcgagaacgccaaagccaagacagaccacggggcggagatcgtgtacaagtcgccagtggtgtctggggacacgtctccacggcatctcagcaatgtctcctccaccggcagcatcgacatggtagactcgccccagctcgccacgctagctgacgaggtgtctgcctccctggccaagcagggtttg

SEQ ID NO: 8 - protein, 410 aa, Homo sapiens
MAEPRQEFEVMEDHAGTYGLGDRKDQGGYTMHQDQEGDTDAGLKESPLQTPTEDGSEEPGSETSDAKSTPTAEDVTAPLVDEGAPGKQAAAQPHTEIPEGTTAEEAGIGDTPSLEDEAAGHVTQARMVSKSKDGTGSDDKKAKGADGKTKIATPRGAAPPGQKGQANATRIPAKTPPAPKTPPSSGEPPKSGDRSGYSSPGSPGTPGSRSRTPSLPTPPTREPKKVAVVRTPPKSPSSAKSRLQTAPVPMPDLKNVKSKIGSTENLKHQPGGGKVQIVYKPVDLSKVTSKCGSLGNIHHKPGGGQVEVKSEKLDFKDRVQSKIGSLDNITHVPGGGNKKIETHKLTFRENAKAKTDHGAEIVYKSPVVSGDTSPRHLSNVSSTGSIDMVDSPQLATLADEVSASLAKQGL

SEQ ID NO: 9 - DNA, 1149 bp, Homo sapiens
  source 1..1149: mol_type = other DNA
  CDS 1..1149
atggctgagccccgccaggagttcgaagtgatggaagatcacgctgggacgtacgggttgggggacaggaaagatcaggggggctacaccatgcaccaagaccaagagggtgacacggacgctggcctgaaagctgaagaagcaggcattggagacacccccagcctggaagacgaagctgctggtcacgtgacccaagctcgcatggtcagtaaaagcaaagacgggactggaagcgatgacaaaaaagccaagggggctgatggtaaaacgaagatcgccacaccgcggggagcagcccctccaggccagaagggccaggccaacgccaccaggattccagcaaaaaccccgcccgctccaaagacaccacccagctctggtgaacctccaaaatcaggggatcgcagcggctacagcagccccggctccccaggcactcccggcagccgctcccgcaccccgtcccttccaaccccacccacccgggagcccaagaaggtggcagtggtccgtactccacccaagtcgccgtcttccgccaagagccgcctgcagacagcccccgtgcccatgccagacctgaagaatgtcaagtccaagatcggctccactgagaacctgaagcaccagccgggaggcgggaaggtgcagataattaataagaagctggatcttagcaacgtccagtccaagtgtggctcaaaggataatatcaaacacgtcccgggaggcggcagtgtgcaaatagtctacaaaccagttgacctgagcaaggtgacctccaagtgtggctcattaggcaacatccatcataaaccaggaggtggccaggtggaagtaaaatctgagaagcttgacttcaaggacagagtccagtcgaagattgggtccctggacaatatcacccacgtccctggcggaggaaataaaaagattgaaacccacaagctgaccttccgcgagaacgccaaagccaagacagaccacggggcggagatcgtgtacaagtcgccagtggtgtctggggacacgtctccacggcatctcagcaatgtctcctccaccggcagcatcgacatggtagactcgccccagctcgccacgctagctgacgaggtgtctgcctccctggccaagcagggtttg

SEQ ID NO: 10 - protein, 383 aa, Homo sapiens
MAEPRQEFEVMEDHAGTYGLGDRKDQGGYTMHQDQEGDTDAGLKAEEAGIGDTPSLEDEAAGHVTQARMVSKSKDGTGSDDKKAKGADGKTKIATPRGAAPPGQKGQANATRIPAKTPPAPKTPPSSGEPPKSGDRSGYSSPGSPGTPGSRSRTPSLPTPPTREPKKVAVVRTPPKSPSSAKSRLQTAPVPMPDLKNVKSKIGSTENLKHQPGGGKVQIINKKLDLSNVQSKCGSKDNIKHVPGGGSVQIVYKPVDLSKVTSKCGSLGNIHHKPGGGQVEVKSEKLDFKDRVQSKIGSLDNITHVPGGGNKKIETHKLTFRENAKAKTDHGAEIVYKSPVVSGDTSPRHLSNVSSTGSIDMVDSPQLATLADEVSASLAKQGL

SEQ ID NO: 11 - DNA, 1236 bp, Homo sapiens
  source 1..1236: mol_type = other DNA
  CDS 1..1236
atggctgagccccgccaggagttcgaagtgatggaagatcacgctgggacgtacgggttgggggacaggaaagatcaggggggctacaccatgcaccaagaccaagagggtgacacggacgctggcctgaaagaatctcccctgcagacccccactgaggacggatctgaggaaccgggctctgaaacctctgatgctaagagcactccaacagcggaagctgaagaagcaggcattggagacacccccagcctggaagacgaagctgctggtcacgtgacccaagctcgcatggtcagtaaaagcaaagacgggactggaagcgatgacaaaaaagccaagggggctgatggtaaaacgaagatcgccacaccgcggggagcagcccctccaggccagaagggccaggccaacgccaccaggattccagcaaaaaccccgcccgctccaaagacaccacccagctctggtgaacctccaaaatcaggggatcgcagcggctacagcagccccggctccccaggcactcccggcagccgctcccgcaccccgtcccttccaaccccacccacccgggagcccaagaaggtggcagtggtccgtactccacccaagtcgccgtcttccgccaagagccgcctgcagacagcccccgtgcccatgccagacctgaagaatgtcaagtccaagatcggctccactgagaacctgaagcaccagccgggaggcgggaaggtgcagataattaataagaagctggatcttagcaacgtccagtccaagtgtggctcaaaggataatatcaaacacgtcccgggaggcggcagtgtgcaaatagtctacaaaccagttgacctgagcaaggtgacctccaagtgtggctcattaggcaacatccatcataaaccaggaggtggccaggtggaagtaaaatctgagaagcttgacttcaaggacagagtccagtcgaagattgggtccctggacaatatcacccacgtccctggcggaggaaataaaaagattgaaacccacaagctgaccttccgcgagaacgccaaagccaagacagaccacggggcggagatcgtgtacaagtcgccagtggtgtctggggacacgtctccacggcatctcagcaatgtctcctccaccggcagcatcgacatggtagactcgccccagctcgccacgctagctgacgaggtgtctgcctccctggccaagcagggtttg

SEQ ID NO: 12 - protein, 412 aa, Homo sapiens
MAEPRQEFEVMEDHAGTYGLGDRKDQGGYTMHQDQEGDTDAGLKESPLQTPTEDGSEEPGSETSDAKSTPTAEAEEAGIGDTPSLEDEAAGHVTQARMVSKSKDGTGSDDKKAKGADGKTKIATPRGAAPPGQKGQANATRIPAKTPPAPKTPPSSGEPPKSGDRSGYSSPGSPGTPGSRSRTPSLPTPPTREPKKVAVVRTPPKSPSSAKSRLQTAPVPMPDLKNVKSKIGSTENLKHQPGGGKVQIINKKLDLSNVQSKCGSKDNIKHVPGGGSVQIVYKPVDLSKVTSKCGSLGNIHHKPGGGQVEVKSEKLDFKDRVQSKIGSLDNITHVPGGGNKKIETHKLTFRENAKAKTDHGAEIVYKSPVVSGDTSPRHLSNVSSTGSIDMVDSPQLATLADEVSASLAKQGL

SEQ ID NO: 13 - DNA, 1323 bp, Homo sapiens
  source 1..1323: mol_type = other DNA
  CDS 1..1323
atggctgagccccgccaggagttcgaagtgatggaagatcacgctgggacgtacgggttgggggacaggaaagatcaggggggctacaccatgcaccaagaccaagagggtgacacggacgctggcctgaaagaatctcccctgcagacccccactgaggacggatctgaggaaccgggctctgaaacctctgatgctaagagcactccaacagcggaagatgtgacagcacccttagtggatgagggagctcccggcaagcaggctgccgcgcagccccacacggagatcccagaaggaaccacagctgaagaagcaggcattggagacacccccagcctggaagacgaagctgctggtcacgtgacccaagctcgcatggtcagtaaaagcaaagacgggactggaagcgatgacaaaaaagccaagggggctgatggtaaaacgaagatcgccacaccgcggggagcagcccctccaggccagaagggccaggccaacgccaccaggattccagcaaaaaccccgcccgctccaaagacaccacccagctctggtgaacctccaaaatcaggggatcgcagcggctacagcagccccggctccccaggcactcccggcagccgctcccgcaccccgtcccttccaaccccacccacccgggagcccaagaaggtggcagtggtccgtactccacccaagtcgccgtcttccgccaagagccgcctgcagacagcccccgtgcccatgccagacctgaagaatgtcaagtccaagatcggctccactgagaacctgaagcaccagccgggaggcgggaaggtgcagataattaataagaagctggatcttagcaacgtccagtccaagtgtggctcaaaggataatatcaaacacgtcccgggaggcggcagtgtgcaaatagtctacaaaccagttgacctgagcaaggtgacctccaagtgtggctcattaggcaacatccatcataaaccaggaggtggccaggtggaagtaaaatctgagaagcttgacttcaaggacagagtccagtcgaagattgggtccctggacaatatcacccacgtccctggcggaggaaataaaaagattgaaacccacaagctgaccttccgcgagaacgccaaagccaagacagaccacggggcggagatcgtgtacaagtcgccagtggtgtctggggacacgtctccacggcatctcagcaatgtctcctccaccggcagcatcgacatggtagactcgccccagctcgccacgctagctgacgaggtgtctgcctccctggccaagcagggtttg

SEQ ID NO: 14 - protein, 441 aa, Homo sapiens
MAEPRQEFEVMEDHAGTYGLGDRKDQGGYTMHQDQEGDTDAGLKESPLQTPTEDGSEEPGSETSDAKSTPTAEDVTAPLVDEGAPGKQAAAQPHTEIPEGTTAEEAGIGDTPSLEDEAAGHVTQARMVSKSKDGTGSDDKKAKGADGKTKIATPRGAAPPGQKGQANATRIPAKTPPAPKTPPSSGEPPKSGDRSGYSSPGSPGTPGSRSRTPSLPTPPTREPKKVAVVRTPPKSPSSAKSRLQTAPVPMPDLKNVKSKIGSTENLKHQPGGGKVQIINKKLDLSNVQSKCGSKDNIKHVPGGGSVQIVYKPVDLSKVTSKCGSLGNIHHKPGGGQVEVKSEKLDFKDRVQSKIGSLDNITHVPGGGNKKIETHKLTFRENAKAKTDHGAEIVYKSPVVSGDTSPRHLSNVSSTGSIDMVDSPQLATLADEVSASLAKQGL

SEQ ID NO: 15 - DNA, 126 bp, Homo sapiens
  source 1..126: mol_type = other DNA
  CDS 1..126
gatgcagaattccgacatgactcaggatatgaagttcatcatcaaaaattggtgttctttgcagaagatgtgggttcaaacaaaggtgcaatcattggactcatggtgggcggtgttgtcatagcg

SEQ ID NO: 16 - protein, 42 aa, Homo sapiens [sequence omitted]

SEQ ID NO: 17 - DNA, 420 bp, Homo sapiens
  source 1..420: mol_type = other DNA
  misc_feature 127..129: note = n is a, c, g, or t
  misc_feature 133..135: note = n is a, c, g, or t
  misc_feature 148..150: note = n is a, c, g, or t
  CDS 1..420
atggatgtattcatgaaaggactttcaaaggccaaggagggagttgtggctgctgctgagaaaaccaaacagggtgtggcagaagcagcaggaaagacaaaagagggtgttctctatgtaggctccnnnaccnnngagggagtggtgnnnggtgtggcaacagtggctgagaagaccaaagagcaagtgacaaatgttggaggagcagtggtgacgggtgtgacagcagtagcccagaagacagtggagggagcagggagcattgcagcagccactggctttgtcaaaaaggaccagttgggcaagaatgaagaaggagccccacaggaaggaattctggaagatatgcctgtggatcctgacaatgaggcttatgaaatgccttctgaggaagggtatcaagactacgaacctgaagcc

SEQ ID NO: 18 - protein, 140 aa, Homo sapiens
  SITE 43: note = misc_feature - The 'X' at location 43 stands for Lys, Asn, Arg, Ser, Thr, Ile, Met, Glu, Asp, Gly, Ala, Val, Gln, His, Pro, Leu, Tyr, Trp, Cys, or Phe, or deletion.
  SITE 45: note = misc_feature - The 'X' at location 45 stands for Lys, Asn, Arg, Ser, Thr, Ile, Met, Glu, Asp, Gly, Ala, Val, Gln, His, Pro, Leu, Tyr, Trp, Cys, or Phe, or deletion.
  SITE 50: note = misc_feature - The 'X' at location 50 stands for Lys, Asn, Arg, Ser, Thr, Ile, Met, Glu, Asp, Gly, Ala, Val, Gln, His, Pro, Leu, Tyr, Trp, Cys, or Phe, or deletion.
MDVFMKGLSKAKEGVVAAAEKTKQGVAEAAGKTKEGVLYVGSXTXEGVVXGVATVAEKTKEQVTNVGGAVVTGVTAVAQKTVEGAGSIAAATGFVKKDQLGKNEEGAPQEGILEDMPVDPDNEAYEMPSEEGYQDYEPEA

SEQ ID NO: 19 - DNA, 1056 bp, Homo sapiens
  source 1..1056: mol_type = other DNA
  misc_feature 718..741: note = n is a, c, g, or t, or deletion.
  CDS 1..1056
atggctgagccccgccaggagttcgaagtgatggaagatcacgctgggacgtacgggttgggggacaggaaagatcaggggggctacaccatgcaccaagaccaagagggtgacacggacgctggcctgaaagctgaagaagcaggcattggagacacccccagcctggaagacgaagctgctggtcacgtgacccaagctcgcatggtcagtaaaagcaaagacgggactggaagcgatgacaaaaaagccaagggggctgatggtaaaacgaagatcgccacaccgcggggagcagcccctccaggccagaagggccaggccaacgccaccaggattccagcaaaaaccccgcccgctccaaagacaccacccagctctggtgaacctccaaaatcaggggatcgcagcggctacagcagccccggctccccaggcactcccggcagccgctcccgcaccccgtcccttccaaccccacccacccgggagcccaagaaggtggcagtggtccgtactccacccaagtcgccgtcttccgccaagagccgcctgcagacagcccccgtgcccatgccagacctgaagaatgtcaagtccaagatcggctccactgagaacctgaagcaccagccgggaggcgggaaggtgcaaatagtctacaaaccagttgacctgagcaaggtgacctccaagtgtggctcattaggcaacatcnnnnnnnnnnnnnnnnnnnnnnnngtggaagtaaaatctgagaagcttgacttcaaggacagagtccagtcgaagattgggtccctggacaatatcacccacgtccctggcggaggaaataaaaagattgaaacccacaagctgaccttccgcgagaacgccaaagccaagacagaccacggggcggagatcgtgtacaagtcgccagtggtgtctggggacacgtctccacggcatctcagcaatgtctcctccaccggcagcatcgacatggtagactcgccccagctcgccacgctagctgacgaggtgtctgcctccctggccaagcagggtttg

SEQ ID NO: 20 - protein, 352 aa, Homo sapiens
  SITE 240: note = misc_feature - The 'X' at location 240 stands for Lys, Asn, Arg, Ser, Thr, Ile, Met, Glu, Asp, Gly, Ala, Val, Gln, His, Pro, Leu, Tyr, Trp, Cys, or Phe.
  SITE 241: note = misc_feature - The 'X' at location 241 stands for Lys, Asn, Arg, Ser, Thr, Ile, Met, Glu, Asp, Gly, Ala, Val, Gln, His, Pro, Leu, Tyr, Trp, Cys, or Phe.
  SITE 242: note = misc_feature - The 'X' at location 242 stands for Lys, or deletion.
  SITE 243: note = misc_feature - The 'X' at location 243 stands for Pro, or deletion.
  SITE 244: note = misc_feature - The 'X' at location 244 stands for Gly, or deletion.
  SITE 245: note = misc_feature - The 'X' at location 245 stands for Gly, or deletion.
  SITE 246: note = misc_feature - The 'X' at location 246 stands for Gly, or deletion.
  SITE 247: note = misc_feature - The 'X' at location 247 stands for Gln, or deletion
MAEPRQEFEVMEDHAGTYGLGDRKDQGGYTMHQDQEGDTDAGLKAEEAGIGDTPSLEDEAAGHVTQARMVSKSKDGTGSDDKKAKGADGKTKIATPRGAAPPGQKGQANATRIPAKTPPAPKTPPSSGEPPKSGDRSGYSSPGSPGTPGSRSRTPSLPTPPTREPKKVAVVRTPPKSPSSAKSRLQTAPVPMPDLKNVKSKIGSTENLKHQPGGGKVQIVYKPVDLSKVTSKCGSLGNIXXXXXXXXVEVKSEKLDFKDRVQSKIGSLDNITHVPGGGNKKIETHKLTFRENAKAKTDHGAEIVYKSPVVSGDTSPRHLSNVSSTGSIDMVDSPQLATLADEVSASLAKQGL

SEQ ID NO: 21 - DNA, 1143 bp, Homo sapiens
  source 1..1143: mol_type = other DNA
  misc_feature 805..828: note = n is a, c, g, or t, or deletion.
  CDS 1..1143
atggctgagccccgccaggagttcgaagtgatggaagatcacgctgggacgtacgggttgggggacaggaaagatcaggggggctacaccatgcaccaagaccaagagggtgacacggacgctggcctgaaagaatctcccctgcagacccccactgaggacggatctgaggaaccgggctctgaaacctctgatgctaagagcactccaacagcggaagctgaagaagcaggcattggagacacccccagcctggaagacgaagctgctggtcacgtgacccaagctcgcatggtcagtaaaagcaaagacgggactggaagcgatgacaaaaaagccaagggggctgatggtaaaacgaagatcgccacaccgcggggagcagcccctccaggccagaagggccaggccaacgccaccaggattccagcaaaaaccccgcccgctccaaagacaccacccagctctggtgaacctccaaaatcaggggatcgcagcggctacagcagccccggctccccaggcactcccggcagccgctcccgcaccccgtcccttccaaccccacccacccgggagcccaagaaggtggcagtggtccgtactccacccaagtcgccgtcttccgccaagagccgcctgcagacagcccccgtgcccatgccagacctgaagaatgtcaagtccaagatcggctccactgagaacctgaagcaccagccgggaggcgggaaggtgcaaatagtctacaaaccagttgacctgagcaaggtgacctccaagtgtggctcattaggcaacatcnnnnnnnnnnnnnnnnnnnnnnnngtggaagtaaaatctgagaagcttgacttcaaggacagagtccagtcgaagattgggtccctggacaatatcacccacgtccctggcggaggaaataaaaagattgaaacccacaagctgaccttccgcgagaacgccaaagccaagacagaccacggggcggagatcgtgtacaagtcgccagtggtgtctggggacacgtctccacggcatctcagcaatgtctcctccaccggcagcatcgacatggtagactcgccccagctcgccacgctagctgacgaggtgtctgcctccctggccaagcagggtttg

SEQ ID NO: 22 - protein, 381 aa, Homo sapiens
  SITE 269: note = misc_feature - The 'X' at location 269 stands for Lys, Asn, Arg, Ser, Thr, Ile, Met, Glu, Asp, Gly, Ala, Val, Gln, His, Pro, Leu, Tyr, Trp, Cys, or Phe.
  SITE 270: note = misc_feature - The 'X' at location 270 stands for Lys, Asn, Arg, Ser, Thr, Ile, Met, Glu, Asp, Gly, Ala, Val, Gln, His, Pro, Leu, Tyr, Trp, Cys, or Phe.
  SITE 271: note = misc_feature - The 'X' at location 271 stands for Lys, or deletion.
  SITE 272: note = misc_feature - The 'X' at location 272 stands for Pro, or deletion.
  SITE 273: note = misc_feature - The 'X' at location 273 stands for Gly, or deletion.
  SITE 274: note = misc_feature - The 'X' at location 274 stands for Gly, or deletion.
  SITE 275: note = misc_feature - The 'X' at location 275 stands for Gly, or deletion.
  SITE 276: note = misc_feature - The 'X' at location 276 stands for Gln, or deletion.
MAEPRQEFEVMEDHAGTYGLGDRKDQGGYTMHQDQEGDTDAGLKESPLQTPTEDGSEEPGSETSDAKSTPTAEAEEAGIGDTPSLEDEAAGHVTQARMVSKSKDGTGSDDKKAKGADGKTKIATPRGAAPPGQKGQANATRIPAKTPPAPKTPPSSGEPPKSGDRSGYSSPGSPGTPGSRSRTPSLPTPPTREPKKVAVVRTPPKSPSSAKSRLQTAPVPMPDLKNVKSKIGSTENLKHQPGGGKVQIVYKPVDLSKVTSKCGSLGNIXXXXXXXXVEVKSEKLDFKDRVQSKIGSLDNITHVPGGGNKKIETHKLTFRENAKAKTDHGAEIVYKSPVVSGDTSPRHLSNVSSTGSIDMVDSPQLATLADEVSASLAKQGL

SEQ ID NO: 23 - DNA, 1230 bp, Homo sapiens
  source 1..1230: mol_type = other DNA
  misc_feature 892..915: note = n is a, c, g, or t, or deletion.
  CDS 1..1230
atggctgagccccgccaggagttcgaagtgatggaagatcacgctgggacgtacgggttgggggacaggaaagatcaggggggctacaccatgcaccaagaccaagagggtgacacggacgctggcctgaaagaatctcccctgcagacccccactgaggacggatctgaggaaccgggctctgaaacctctgatgctaagagcactccaacagcggaagatgtgacagcacccttagtggatgagggagctcccggcaagcaggctgccgcgcagccccacacggagatcccagaaggaaccacagctgaagaagcaggcattggagacacccccagcctggaagacgaagctgctggtcacgtgacccaagctcgcatggtcagtaaaagcaaagacgggactggaagcgatgacaaaaaagccaagggggctgatggtaaaacgaagatcgccacaccgcggggagcagcccctccaggccagaagggccaggccaacgccaccaggattccagcaaaaaccccgcccgctccaaagacaccacccagctctggtgaacctccaaaatcaggggatcgcagcggctacagcagccccggctccccaggcactcccggcagccgctcccgcaccccgtcccttccaaccccacccacccgggagcccaagaaggtggcagtggtccgtactccacccaagtcgccgtcttccgccaagagccgcctgcagacagcccccgtgcccatgccagacctgaagaatgtcaagtccaagatcggctccactgagaacctgaagcaccagccgggaggcgggaaggtgcaaatagtctacaaaccagttgacctgagcaaggtgacctccaagtgtggctcattaggcaacatcnnnnnnnnnnnnnnnnnnnnnnnngtggaagtaaaatctgagaagcttgacttcaaggacagagtccagtcgaagattgggtccctggacaatatcacccacgtccctggcggaggaaataaaaagattgaaacccacaagctgaccttccgcgagaacgccaaagccaagacagaccacggggcggagatcgtgtacaagtcgccagtggtgtctggggacacgtctccacggcatctcagcaatgtctcctccaccggcagcatcgacatggtagactcgccccagctcgccacgctagctgacgaggtgtctgcctccctggccaagcagggtttg

SEQ ID NO: 24 - protein, 410 aa, Homo sapiens
  SITE 298: note = misc_feature - The 'X' at location 298 stands for Lys, Asn, Arg, Ser, Thr, Ile, Met, Glu, Asp, Gly, Ala, Val, Gln, His, Pro, Leu, Tyr, Trp, Cys, or Phe.
  SITE 299: note = misc_feature - The 'X' at location 299 stands for Lys, Asn, Arg, Ser, Thr, Ile, Met, Glu, Asp, Gly, Ala, Val, Gln, His, Pro, Leu, Tyr, Trp, Cys, or Phe.
  SITE 300: note = misc_feature - The 'X' at location 300 stands for Lys, or deletion.
  SITE 301: note = misc_feature - The 'X' at location 301 stands for Pro, or deletion.
  SITE 302: note = misc_feature - The 'X' at location 302 stands for Gly, or deletion.
  SITE 303: note = misc_feature - The 'X' at location 303 stands for Gly, or deletion.
  SITE 304: note = misc_feature - The 'X' at location 304 stands for Gly, or deletion.
  SITE 305: note = misc_feature - The 'X' at location 305 stands for Gln, or deletion.
MAEPRQEFEVMEDHAGTYGLGDRKDQGGYTMHQDQEGDTDAGLKESPLQTPTEDGSEEPGSETSDAKSTPTAEDVTAPLVDEGAPGKQAAAQPHTEIPEGTTAEEAGIGDTPSLEDEAAGHVTQARMVSKSKDGTGSDDKKAKGADGKTKIATPRGAAPPGQKGQANATRIPAKTPPAPKTPPSSGEPPKSGDRSGYSSPGSPGTPGSRSRTPSLPTPPTREPKKVAVVRTPPKSPSSAKSRLQTAPVPMPDLKNVKSKIGSTENLKHQPGGGKVQIVYKPVDLSKVTSKCGSLGNIXXXXXXXXVEVKSEKLDFKDRVQSKIGSLDNITHVPGGGNKKIETHKLTFRENAKAKTDHGAEIVYKSPVVSGDTSPRHLSNVSSTGSIDMVDSPQLATLADEVSASLAKQGL

SEQ ID NO: 25 - DNA, 1149 bp, Homo sapiens
  source 1..1149: mol_type = other DNA
  misc_feature 811..834: note = n is a, c, g, or t, or deletion.
  CDS 1..1149
atggctgagccccgccaggagttcgaagtgatggaagatcacgctgggacgtacgggttgggggacaggaaagatcaggggggctacaccatgcaccaagaccaagagggtgacacggacgctggcctgaaagctgaagaagcaggcattggagacacccccagcctggaagacgaagctgctggtcacgtgacccaagctcgcatggtcagtaaaagcaaagacgggactggaagcgatgacaaaaaagccaagggggctgatggtaaaacgaagatcgccacaccgcggggagcagcccctccaggccagaagggccaggccaacgccaccaggattccagcaaaaaccccgcccgctccaaagacaccacccagctctggtgaacctccaaaatcaggggatcgcagcggctacagcagccccggctccccaggcactcccggcagccgctcccgcaccccgtcccttccaaccccacccacccgggagcccaagaaggtggcagtggtccgtactccacccaagtcgccgtcttccgccaagagccgcctgcagacagcccccgtgcccatgccagacctgaagaatgtcaagtccaagatcggctccactgagaacctgaagcaccagccgggaggcgggaaggtgcagataattaataagaagctggatcttagcaacgtccagtccaagtgtggctcaaaggataatatcaaacacgtcccgggaggcggcagtgtgcaaatagtctacaaaccagttgacctgagcaaggtgacctccaagtgtggctcattaggcaacatcnnnnnnnnnnnnnnnnnnnnnnnngtggaagtaaaatctgagaagcttgacttcaaggacagagtccagtcgaagattgggtccctggacaatatcacccacgtccctggcggaggaaataaaaagattgaaacccacaagctgaccttccgcgagaacgccaaagccaagacagaccacggggcggagatcgtgtacaagtcgccagtggtgtctggggacacgtctccacggcatctcagcaatgtctcctccaccggcagcatcgacatggtagactcgccccagctcgccacgctagctgacgaggtgtctgcctccctggccaagcagggtttg

SEQ ID NO: 26 - protein, 383 aa, Homo sapiens
  SITE 271: note = misc_feature - The 'X' at location 271 stands for Lys, Asn, Arg, Ser, Thr, Ile, Met, Glu, Asp, Gly, Ala, Val, Gln, His, Pro, Leu, Tyr, Trp, Cys, or Phe.
  SITE 272: note = misc_feature - The 'X' at location 272 stands for Lys, Asn, Arg, Ser, Thr, Ile, Met, Glu, Asp, Gly, Ala, Val, Gln, His, Pro, Leu, Tyr, Trp, Cys, or Phe.
  SITE 273: note = misc_feature - The 'X' at location 273 stands for Lys, or deletion.
  SITE 274: note = misc_feature - The 'X' at location 274 stands for Pro, or deletion.
  SITE 275: note = misc_feature - The 'X' at location 275 stands for Gly, or deletion.
  SITE 276: note = misc_feature - The 'X' at location 276 stands for Gly, or deletion.
  SITE 277: note = misc_feature - The 'X' at location 277 stands for Gly, or deletion.
  SITE 278: note = misc_feature - The 'X' at location 278 stands for Gln, or deletion.
MAEPRQEFEVMEDHAGTYGLGDRKDQGGYTMHQDQEGDTDAGLKAEEAGIGDTPSLEDEAAGHVTQARMVSKSKDGTGSDDKKAKGADGKTKIATPRGAAPPGQKGQANATRIPAKTPPAPKTPPSSGEPPKSGDRSGYSSPGSPGTPGSRSRTPSLPTPPTREPKKVAVVRTPPKSPSSAKSRLQTAPVPMPDLKNVKSKIGSTENLKHQPGGGKVQIINKKLDLSNVQSKCGSKDNIKHVPGGGSVQIVYKPVDLSKVTSKCGSLGNIXXXXXXXXVEVKSEKLDFKDRVQSKIGSLDNITHVPGGGNKKIETHKLTFRENAKAKTDHGAEIVYKSPVVSGDTSPRHLSNVSSTGSIDMVDSPQLATLADEVSASLAKQGL

SEQ ID NO: 27 - DNA, 1236 bp, Homo sapiens
  source 1..1236: mol_type = other DNA
  misc_feature 898..921: note = n is a, c, g, or t, or deletion.
  CDS 1..1236
atggctgagccccgccaggagttcgaagtgatggaagatcacgctgggacgtacgggttgggggacaggaaagatcaggggggctacaccatgcaccaagaccaagagggtgacacggacgctggcctgaaagaatctcccctgcagacccccactgaggacggatctgaggaaccgggctctgaaacctctgatgctaagagcactccaacagcggaagctgaagaagcaggcattggagacacccccagcctggaagacgaagctgctggtcacgtgacccaagctcgcatggtcagtaaaagcaaagacgggactggaagcgatgacaaaaaagccaagggggctgatggtaaaacgaagatcgccacaccgcggggagcagcccctccaggccagaagggccaggccaacgccaccaggattccagcaaaaaccccgcccgctccaaagacaccacccagctctggtgaacctccaaaatcaggggatcgcagcggctacagcagccccggctccccaggcactcccggcagccgctcccgcaccccgtcccttccaaccccacccacccgggagcccaagaaggtggcagtggtccgtactccacccaagtcgccgtcttccgccaagagccgcctgcagacagcccccgtgcccatgccagacctgaagaatgtcaagtccaagatcggctccactgagaacctgaagcaccagccgggaggcgggaaggtgcagataattaataagaagctggatcttagcaacgtccagtccaagtgtggctcaaaggataatatcaaacacgtcccgggaggcggcagtgtgcaaatagtctacaaaccagttgacctgagcaaggtgacctccaagtgtggctcattaggcaacatcnnnnnnnnnnnnnnnnnnnnnnnngtggaagtaaaatctgagaagcttgacttcaaggacagagtccagtcgaagattgggtccctggacaatatcacccacgtccctggcggaggaaataaaaagattgaaacccacaagctgaccttccgcgagaacgccaaagccaagacagaccacggggcggagatcgtgtacaagtcgccagtggtgtctggggacacgtctccacggcatctcagcaatgtctcctccaccggcagcatcgacatggtagactcgccccagctcgccacgctagctgacgaggtgtctgcctccctggccaagcagggtttg

SEQ ID NO: 28 - protein, 412 aa, Homo sapiens
  SITE 300: note = misc_feature - The 'X' at location 300 stands for Lys, Asn, Arg, Ser, Thr, Ile, Met, Glu, Asp, Gly, Ala, Val, Gln, His, Pro, Leu, Tyr, Trp, Cys, or Phe.
  SITE 301: note = misc_feature - The 'X' at location 301 stands for Lys, Asn, Arg, Ser, Thr, Ile, Met, Glu, Asp, Gly, Ala, Val, Gln, His, Pro, Leu, Tyr, Trp, Cys, or Phe.
  SITE 302: note = misc_feature - The 'X' at location 302 stands for Lys, or deletion.
  SITE 303: note = misc_feature - The 'X' at location 303 stands for Pro, or deletion.
  SITE 304: note = misc_feature - The 'X' at location 304 stands for Gly, or deletion.
  SITE 305: note = misc_feature - The 'X' at location 305 stands for Gly, or deletion.
  SITE 306: note = misc_feature - The 'X' at location 306 stands for Gly, or deletion.
  SITE 307: note = misc_feature - The 'X' at location 307 stands for Gln, or deletion.
MAEPRQEFEVMEDHAGTYGLGDRKDQGGYTMHQDQEGDTDAGLKESPLQTPTEDGSEEPGSETSDAKSTPTAEAEEAGIGDTPSLEDEAAGHVTQARMVSKSKDGTGSDDKKAKGADGKTKIATPRGAAPPGQKGQANATRIPAKTPPAPKTPPSSGEPPKSGDRSGYSSPGSPGTPGSRSRTPSLPTPPTREPKKVAVVRTPPKSPSSAKSRLQTAPVPMPDLKNVKSKIGSTENLKHQPGGGKVQIINKKLDLSNVQSKCGSKDNIKHVPGGGSVQIVYKPVDLSKVTSKCGSLGNIXXXXXXXXVEVKSEKLDFKDRVQSKIGSLDNITHVPGGGNKKIETHKLTFRENAKAKTDHGAEIVYKSPVVSGDTSPRHLSNVSSTGSIDMVDSPQLATLADEVSASLAKQGL

SEQ ID NO: 29 - DNA, 1323 bp, Homo sapiens
  source 1..1323: mol_type = other DNA
  misc_feature 985..1008: note = n is a, c, g, or t, or deletion.
  CDS 1..1323
atggctgagccccgccaggagttcgaagtgatggaagatcacgctgggacgtacgggttgggggacaggaaagatcaggggggctacaccatgcaccaagaccaagagggtgacacggacgctggcctgaaagaatctcccctgcagacccccactgaggacggatctgaggaaccgggctctgaaacctctgatgctaagagcactccaacagcggaagatgtgacagcacccttagtggatgagggagctcccggcaagcaggctgccgcgcagccccacacggagatcccagaaggaaccacagctgaagaagcaggcattggagacacccccagcctggaagacgaagctgctggtcacgtgacccaagctcgcatggtcagtaaaagcaaagacgggactggaagcgatgacaaaaaagccaagggggctgatggtaaaacgaagatcgccacaccgcggggagcagcccctccaggccagaagggccaggccaacgccaccaggattccagcaaaaaccccgcccgctccaaagacaccacccagctctggtgaacctccaaaatcaggggatcgcagcggctacagcagccccggctccccaggcactcccggcagccgctcccgcaccccgtcccttccaaccccacccacccgggagcccaagaaggtggcagtggtccgtactccacccaagtcgccgtcttccgccaagagccgcctgcagacagcccccgtgcccatgccagacctgaagaatgtcaagtccaagatcggctccactgagaacctgaagcaccagccgggaggcgggaaggtgcagataattaataagaagctggatcttagcaacgtccagtccaagtgtggctcaaaggataatatcaaacacgtcccgggaggcggcagtgtgcaaatagtctacaaaccagttgacctgagcaaggtgacctccaagtgtggctcattaggcaacatcnnnnnnnnnnnnnnnnnnnnnnnngtggaagtaaaatctgagaagcttgacttcaaggacagagtccagtcgaagattgggtccctggacaatatcacccacgtccctggcggaggaaataaaaagattgaaacccacaagctgaccttccgcgagaacgccaaagccaagacagaccacggggcggagatcgtgtacaagtcgccagtggtgtctggggacacgtctccacggcatctcagcaatgtctcctccaccggcagcatcgacatggtagactcgccccagctcgccacgctagctgacgaggtgtctgcctccctggccaagcagggtttg

SEQ ID NO: 30 - protein, 441 aa, Homo sapiens
  SITE 329: note = misc_feature - The 'X' at location 329 stands for Lys, Asn, Arg, Ser, Thr, Ile, Met, Glu, Asp, Gly, Ala, Val, Gln, His, Pro, Leu, Tyr, Trp, Cys, or Phe.
  SITE 330: note = misc_feature - The 'X' at location 330 stands for Lys, Asn, Arg, Ser, Thr, Ile, Met, Glu, Asp, Gly, Ala, Val, Gln, His, Pro, Leu, Tyr, Trp, Cys, or Phe.
  SITE 331: note = misc_feature - The 'X' at location 331 stands for Lys, or deletion.
  SITE 332: note = misc_feature - The 'X' at location 332 stands for Pro, or deletion.
  SITE 333: note = misc_feature - The 'X' at location 333 stands for Gly, or deletion.
  SITE 334: note = misc_feature - The 'X' at location 334 stands for Gly, or deletion.
  SITE 335: note = misc_feature - The 'X' at location 335 stands for Gly, or deletion.
  SITE 336: note = misc_feature - The 'X' at location 336 stands for Gln, or deletion.
MAEPRQEFEVMEDHAGTYGLGDRKDQGGYTMHQDQEGDTDAGLKESPLQTPTEDGSEEPGSETSDAKSTPTAEDVTAPLVDEGAPGKQAAAQPHTEIPEGTTAEEAGIGDTPSLEDEAAGHVTQARMVSKSKDGTGSDDKKAKGADGKTKIATPRGAAPPGQKGQANATRIPAKTPPAPKTPPSSGEPPKSGDRSGYSSPGSPGTPGSRSRTPSLPTPPTREPKKVAVVRTPPKSPSSAKSRLQTAPVPMPDLKNVKSKIGSTENLKHQPGGGKVQIINKKLDLSNVQSKCGSKDNIKHVPGGGSVQIVYKPVDLSKVTSKCGSLGNIXXXXXXXXVEVKSEKLDFKDRVQSKIGSLDNITHVPGGGNKKIETHKLTFRENAKAKTDHGAEIVYKSPVVSGDTSPRHLSNVSSTGSIDMVDSPQLATLADEVSASLAKQGL

SEQ ID NO: 31 - DNA, 126 bp, Homo sapiens
  source 1..126: mol_type = other DNA
  misc_feature 82..84: note = n is a, c, g, or t, or deletion.
  misc_feature 100..102: note = n is a, c, g, or t, or deletion.
  misc_feature 106..108: note = n is a, c, g, or t, or deletion.
  CDS 1..126
gatgcagaattccgacatgactcaggatatgaagttcatcatcaaaaattggtgttctttgcagaagatgtgggttcaaacnnnggtgcaatcattggannnatgnnnggcggtgttgtcatagcg

SEQ ID NO: 32 - protein, 42 aa, Homo sapiens
  SITE 28: note = misc_feature - The 'X' at location 28 stands for Lys, Asn, Arg, Ser, Thr, Ile, Met, Glu, Asp, Gly, Ala, Val, Gln, His, Pro, Leu, Tyr, Trp, Cys, or Phe, or deletion.
  SITE 34: note = misc_feature - The 'X' at location 34 stands for Lys, Asn, Arg, Ser, Thr, Ile, Met, Glu, Asp, Gly, Ala, Val, Gln, His, Pro, Leu, Tyr, Trp, Cys, or Phe, or deletion.
  SITE 36: note = misc_feature - The 'X' at location 36 stands for Lys, Asn, Arg, Ser, Thr, Ile, Met, Glu, Asp, Gly, Ala, Val, Gln, His, Pro, Leu, Tyr, Trp, Cys, or Phe, or deletion.
DAEFRHDSGYEVHHQKLVFFAEDVGSNXGAIIGXMXGGVVIA

SEQ ID NO: 33 - DNA, 420 bp, Homo sapiens; identical to SEQ ID NO: 17
  source 1..420: mol_type = other DNA
  misc_feature 127..129: note = n is a, c, g, or t
  misc_feature 133..135: note = n is a, c, g, or t
  misc_feature 148..150: note = n is a, c, g, or t
  CDS 1..420

SEQ ID NO: 34 - protein, 140 aa, Homo sapiens; identical to SEQ ID NO: 18
  SITE 43: note = misc_feature - The 'X' at location 43 stands for Lys, Asn, Arg, Ser, Thr, Ile, Met, Glu, Asp, Gly, Ala, Val, Gln, His, Pro, Leu, Tyr, Trp, Cys, or Phe.
  SITE 45: note = misc_feature - The 'X' at location 45 stands for Lys, Asn, Arg, Ser, Thr, Ile, Met, Glu, Asp, Gly, Ala, Val, Gln, His, Pro, Leu, Tyr, Trp, Cys, or Phe.
  SITE 50: note = misc_feature - The 'X' at location 50 stands for Lys, Asn, Arg, Ser, Thr, Ile, Met, Glu, Asp, Gly, Ala, Val, Gln, His, Pro, Leu, Tyr, Trp, Cys, or Phe.

SEQ ID NO: 35 - DNA, 1056 bp, Homo sapiens
  source 1..1056: mol_type = other DNA
  misc_feature 718..726: note = n is a, c, g, or t
  CDS 1..1056
atggctgagccccgccaggagttcgaagtgatggaagatcacgctgggacgtacgggttgggggacaggaaagatcaggggggctacaccatgcaccaagaccaagagggtgacacggacgctggcctgaaagctgaagaagcaggcattggagacacccccagcctggaagacgaagctgctggtcacgtgacccaagctcgcatggtcagtaaaagcaaagacgggactggaagcgatgacaaaaaagccaagggggctgatggtaaaacgaagatcgccacaccgcggggagcagcccctccaggccagaagggccaggccaacgccaccaggattccagcaaaaaccccgcccgctccaaagacaccacccagctctggtgaacctccaaaatcaggggatcgcagcggctacagcagccccggctccccaggcactcccggcagccgctcccgcaccccgtcccttccaaccccacccacccgggagcccaagaaggtggcagtggtccgtactccacccaagtcgccgtcttccgccaagagccgcctgcagacagcccccgtgcccatgccagacctgaagaatgtcaagtccaagatcggctccactgagaacctgaagcaccagccgggaggcgggaaggtgcaaatagtctacaaaccagttgacctgagcaaggtgacctccaagtgtggctcattaggcaacatcnnnnnnnnnccaggaggtggccaggtggaagtaaaatctgagaagcttgacttcaaggacagagtccagtcgaagattgggtccctggacaatatcacccacgtccctggcggaggaaataaaaagattgaaacccacaagctgaccttccgcgagaacgccaaagccaagacagaccacggggcggagatcgtgtacaagtcgccagtggtgtctggggacacgtctccacggcatctcagcaatgtctcctccaccggcagcatcgacatggtagactcgccccagctcgccacgctagctgacgaggtgtctgcctccctggccaagcagggtttg

SEQ ID NO: 36 - protein, 352 aa, Homo sapiens
  SITE 240: note = misc_feature - The 'X' at location 240 stands for Lys, Asn, Arg, Ser, Thr, Ile, Met, Glu, Asp, Gly, Ala, Val, Gln, His, Pro, Leu, Tyr, Trp, Cys, or Phe.
  SITE 241: note = misc_feature - The 'X' at location 241 stands for Lys, Asn, Arg, Ser, Thr, Ile, Met, Glu, Asp, Gly, Ala, Val, Gln, His, Pro, Leu, Tyr, Trp, Cys, or Phe.
  SITE 242: note = misc_feature - The 'X' at location 242 stands for Lys, Asn, Arg, Ser, Thr, Ile, Met, Glu, Asp, Gly, Ala, Val, Gln, His, Pro, Leu, Tyr, Trp, Cys, or Phe.
MAEPRQEFEVMEDHAGTYGLGDRKDQGGYTMHQDQEGDTDAGLKAEEAGIGDTPSLEDEAAGHVTQARMVSKSKDGTGSDDKKAKGADGKTKIATPRGAAPPGQKGQANATRIPAKTPPAPKTPPSSGEPPKSGDRSGYSSPGSPGTPGSRSRTPSLPTPPTREPKKVAVVRTPPKSPSSAKSRLQTAPVPMPDLKNVKSKIGSTENLKHQPGGGKVQIVYKPVDLSKVTSKCGSLGNIXXXPGGGQVEVKSEKLDFKDRVQSKIGSLDNITHVPGGGNKKIETHKLTFRENAKAKTDHGAEIVYKSPVVSGDTSPRHLSNVSSTGSIDMVDSPQLATLADEVSASLAKQGL

SEQ ID NO: 37 - DNA, 1143 bp, Homo sapiens
  source 1..1143: mol_type = other DNA
  misc_feature 805..813: note = n is a, c, g, or t
  CDS 1..1143
atggctgagccccgccaggagttcgaagtgatggaagatcacgctgggacgtacgggttgggggacaggaaagatcaggggggctacaccatgcaccaagaccaagagggtgacacggacgctggcctgaaagaatctcccctgcagacccccactgaggacggatctgaggaaccgggctctgaaacctctgatgctaagagcactccaacagcggaagctgaagaagcaggcattggagacacccccagcctggaagacgaagctgctggtcacgtgacccaagctcgcatggtcagtaaaagcaaagacgggactggaagcgatgacaaaaaagccaagggggctgatggtaaaacgaagatcgccacaccgcggggagcagcccctccaggccagaagggccaggccaacgccaccaggattccagcaaaaaccccgcccgctccaaagacaccacccagctctggtgaacctccaaaatcaggggatcgcagcggctacagcagccccggctccccaggcactcccggcagccgctcccgcaccccgtcccttccaaccccacccacccgggagcccaagaaggtggcagtggtccgtactccacccaagtcgccgtcttccgccaagagccgcctgcagacagcccccgtgcccatgccagacctgaagaatgtcaagtccaagatcggctccactgagaacctgaagcaccagccgggaggcgggaaggtgcaaatagtctacaaaccagttgacctgagcaaggtgacctccaagtgtggctcattaggcaacatcnnnnnnnnnccaggaggtggccaggtggaagtaaaatctgagaagcttgacttcaaggacagagtccagtcgaagattgggtccctggacaatatcacccacgtccctggcggaggaaataaaaagattgaaacccacaagctgaccttccgcgagaacgccaaagccaagacagaccacggggcggagatcgtgtacaagtcgccagtggtgtctggggacacgtctccacggcatctcagcaatgtctcctccaccggcagcatcgacatggtagactcgccccagctcgccacgctagctgacgaggtgtctgcctccctggccaagcagggtttg

SEQ ID NO: 38 - protein, 381 aa, Homo sapiens
  SITE 269: note = misc_feature - The 'X' at location 269 stands for Lys, Asn, Arg, Ser, Thr, Ile, Met, Glu, Asp, Gly, Ala, Val, Gln, His, Pro, Leu, Tyr, Trp, Cys, or Phe.
  SITE 270: note = misc_feature - The 'X' at location 270 stands for Lys, Asn, Arg, Ser, Thr, Ile, Met, Glu, Asp, Gly, Ala, Val, Gln, His, Pro, Leu, Tyr, Trp, Cys, or Phe.
  SITE 271: note = misc_feature - The 'X' at location 271 stands for Lys, Asn, Arg, Ser, Thr, Ile, Met, Glu, Asp, Gly, Ala, Val, Gln, His, Pro, Leu, Tyr, Trp, Cys, or Phe.
MAEPRQEFEVMEDHAGTYGLGDRKDQGGYTMHQDQEGDTDAGLKESPLQTPTEDGSEEPGSETSDAKSTPTAEAEEAGIGDTPSLEDEAAGHVTQARMVSKSKDGTGSDDKKAKGADGKTKIATPRGAAPPGQKGQANATRIPAKTPPAPKTPPSSGEPPKSGDRSGYSSPGSPGTPGSRSRTPSLPTPPTREPKKVAVVRTPPKSPSSAKSRLQTAPVPMPDLKNVKSKIGSTENLKHQPGGGKVQIVYKPVDLSKVTSKCGSLGNIXXXPGGGQVEVKSEKLDFKDRVQSKIGSLDNITHVPGGGNKKIETHKLTFRENAKAKTDHGAEIVYKSPVVSGDTSPRHLSNVSSTGSIDMVDSPQLATLADEVSASLAKQGL

SEQ ID NO: 39 - DNA, 1230 bp, Homo sapiens
  source 1..1230: mol_type = other DNA
  misc_feature 892..900: note = n is a, c, g, or t
  CDS 1..1230
atggctgagccccgccaggagttcgaagtgatggaagatcacgctgggacgtacgggttgggggacaggaaagatcaggggggctacaccatgcaccaagaccaagagggtgacacggacgctggcctgaaagaatctcccctgcagacccccactgaggacggatctgaggaaccgggctctgaaacctctgatgctaagagcactccaacagcggaagatgtgacagcacccttagtggatgagggagctcccggcaagcaggctgccgcgcagccccacacggagatcccagaaggaaccacagctgaagaagcaggcattggagacacccccagcctggaagacgaagctgctggtcacgtgacccaagctcgcatggtcagtaaaagcaaagacgggactggaagcgatgacaaaaaagccaagggggctgatggtaaaacgaagatcgccacaccgcggggagcagcccctccaggccagaagggccaggccaacgccaccaggattccagcaaaaaccccgcccgctccaaagacaccacccagctctggtgaacctccaaaatcaggggatcgcagcggctacagcagccccggctccccaggcactcccggcagccgctcccgcaccccgtcccttccaaccccacccacccgggagcccaagaaggtggcagtggtccgtactccacccaagtcgccgtcttccgccaagagccgcctgcagacagcccccgtgcccatgccagacctgaagaatgtcaagtccaagatcggctccactgagaacctgaagcaccagccgggaggcgggaaggtgcaaatagtctacaaaccagttgacctgagcaaggtgacctccaagtgtggctcattaggcaacatcnnnnnnnnnccaggaggtggccaggtggaagtaaaatctgagaagcttgacttcaaggacagagtccagtcgaagattgggtccctggacaatatcacccacgtccctggcggaggaaataaaaagattgaaacccacaagctgaccttccgcgagaacgccaaagccaagacagaccacggggcggagatcgtgtacaagtcgccagtggtgtctggggacacgtctccacggcatctcagcaatgtctcctccaccggcagcatcgacatggtagactcgccccagctcgccacgctagctgacgaggtgtctgcctccctggccaagcagggtttg

SEQ ID NO: 40 - protein, 410 aa, Homo sapiens
  SITE 298: note = misc_feature - The 'X' at location 298 stands for Lys, Asn, Arg, Ser, Thr, Ile, Met, Glu, Asp, Gly, Ala, Val, Gln, His, Pro, Leu, Tyr, Trp, Cys, or Phe.
  SITE 299: note = misc_feature - The 'X' at location 299 stands for Lys, Asn, Arg, Ser, Thr, Ile, Met, Glu, Asp, Gly, Ala, Val, Gln, His, Pro, Leu, Tyr, Trp, Cys, or Phe.
  SITE 300: note = misc_feature - The 'X' at location 300 stands for Lys, Asn, Arg, Ser, Thr, Ile, Met, Glu, Asp, Gly, Ala, Val, Gln, His, Pro, Leu, Tyr, Trp, Cys, or Phe.
MAEPRQEFEVMEDHAGTYGLGDRKDQGGYTMHQDQEGDTDAGLKESPLQTPTEDGSEEPGSETSDAKSTPTAEDVTAPLVDEGAPGKQAAAQPHTEIPEGTTAEEAGIGDTPSLEDEAAGHVTQARMVSKSKDGTGSDDKKAKGADGKTKIATPRGAAPPGQKGQANATRIPAKTPPAPKTPPSSGEPPKSGDRSGYSSPGSPGTPGSRSRTPSLPTPPTREPKKVAVVRTPPKSPSSAKSRLQTAPVPMPDLKNVKSKIGSTENLKHQPGGGKVQIVYKPVDLSKVTSKCGSLGNIXXXPGGGQVEVKSEKLDFKDRVQSKIGSLDNITHVPGGGNKKIETHKLTFRENAKAKTDHGAEIVYKSPVVSGDTSPRHLSNVSSTGSIDMVDSPQLATLADEVSASLAKQGL

SEQ ID NO: 41 - DNA, 1149 bp, Homo sapiens
  source 1..1149: mol_type = other DNA
  misc_feature 811..819: note = n is a, c, g, or t
  CDS 1..1149
atggctgagccccgccaggagttcgaagtgatggaagatcacgctgggacgtacgggttgggggacaggaaagatcaggggggctacaccatgcaccaagaccaagagggtgacacggacgctggcctgaaagctgaagaagcaggcattggagacacccccagcctggaagacgaagctgctggtcacgtgacccaagctcgcatggtcagtaaaagcaaagacgggactggaagcgatgacaaaaaagccaagggggctgatggtaaaacgaagatcgccacaccgcggggagcagcccctccaggccagaagggccaggccaacgccaccaggattccagcaaaaaccccgcccgctccaaagacaccacccagctctggtgaacctccaaaatcaggggatcgcagcggctacagcagccccggctccccaggcactcccggcagccgctcccgcaccccgtcccttccaaccccacccacccgggagcccaagaaggtggcagtggtccgtactccacccaagtcgccgtcttccgccaagagccgcctgcagacagcccccgtgcccatgccagacctgaagaatgtcaagtccaagatcggctccactgagaacctgaagcaccagccgggaggcgggaaggtgcagataattaataagaagctggatcttagcaacgtccagtccaagtgtggctcaaaggataatatcaaacacgtcccgggaggcggcagtgtgcaaatagtctacaaaccagttgacctgagcaaggtgacctccaagtgtggctcattaggcaacatcnnnnnnnnnccaggaggtggccaggtggaagtaaaatctgagaagcttgacttcaaggacagagtccagtcgaagattgggtccctggacaatatcacccacgtccctggcggaggaaataaaaagattgaaacccacaagctgaccttccgcgagaacgccaaagccaagacagaccacggggcggagatcgtgtacaagtcgccagtggtgtctggggacacgtctccacggcatctcagcaatgtctcctccaccggcagcatcgacatggtagactcgccccagctcgccacgctagctgacgaggtgtctgcctccctggccaagcagggtttg

SEQ ID NO: 42 - protein, 383 aa, Homo sapiens
  SITE 271: note = misc_feature - The 'X' at location 271 stands for Lys, Asn, Arg, Ser, Thr, Ile, Met, Glu, Asp, Gly, Ala, Val, Gln, His, Pro, Leu, Tyr, Trp, Cys, or Phe.
  SITE 272: note = misc_feature - The 'X' at location 272 stands for Lys, Asn, Arg, Ser, Thr, Ile, Met, Glu, Asp, Gly, Ala, Val, Gln, His, Pro, Leu, Tyr, Trp, Cys, or Phe.
  SITE 273: note = misc_feature - The 'X' at location 273 stands for Lys, Asn, Arg, Ser, Thr, Ile, Met, Glu, Asp, Gly, Ala, Val, Gln, His, Pro, Leu, Tyr, Trp, Cys, or Phe.
MAEPRQEFEVMEDHAGTYGLGDRKDQGGYTMHQDQEGDTDAGLKAEEAGIGDTPSLEDEAAGHVTQARMVSKSKDGTGSDDKKAKGADGKTKIATPRGAAPPGQKGQANATRIPAKTPPAPKTPPSSGEPPKSGDRSGYSSPGSPGTPGSRSRTPSLPTPPTREPKKVAVVRTPPKSPSSAKSRLQTAPVPMPDLKNVKSKIGSTENLKHQPGGGKVQIINKKLDLSNVQSKCGSKDNIKHVPGGGSVQIVYKPVDLSKVTSKCGSLGNIXXXPGGGQVEVKSEKLDFKDRVQSKIGSLDNITHVPGGGNKKIETHKLTFRENAKAKTDHGAEIVYKSPVVSGDTSPRHLSNVSSTGSIDMVDSPQLATLADEVSASLAKQGL

SEQ ID NO: 43 - DNA, 1236 bp, Homo sapiens
  source 1..1236: mol_type = other DNA
  misc_feature 898..906: note = n is a, c, g, or t
  CDS 1..1236
atggctgagccccgccaggagttcgaagtgatggaagatcacgctgggacgtacgggttgggggacaggaaagatcaggggggctacaccatgcaccaagaccaagagggtgacacggacgctggcctgaaagaatctcccctgcagacccccactgaggacggatctgaggaaccgggctctgaaacctctgatgctaagagcactccaacagcggaagctgaagaagcaggcattggagacacccccagcctggaagacgaagctgctggtcacgtgacccaagctcgcatggtcagtaaaagcaaagacgggactggaagcgatgacaaaaaagccaagggggctgatggtaaaacgaagatcgccacaccgcggggagcagcccctccaggccagaagggccaggccaacgccaccaggattccagcaaaaaccccgcccgctccaaagacaccacccagctctggtgaacctccaaaatcaggggatcgcagcggctacagcagccccggctccccaggcactcccggcagccgctcccgcaccccgtcccttccaaccccacccacccgggagcccaagaaggtggcagtggtccgtactccacccaagtcgccgtcttccgccaagagccgcctgcagacagcccccgtgcccatgccagacctgaagaatgtcaagtccaagatcggctccactgagaacctgaagcaccagccgggaggcgggaaggtgcagataattaataagaagctggatcttagcaacgtccagtccaagtgtggctcaaaggataatatcaaacacgtcccgggaggcggcagtgtgcaaatagtctacaaaccagttgacctgagcaaggtgacctccaagtgtggctcattaggcaacatcnnnnnnnnnccaggaggtggccaggtggaagtaaaatctgagaagcttgacttcaaggacagagtccagtcgaagattgggtccctggacaatatcacccacgtccctggcggaggaaataaaaagattgaaacccacaagctgaccttccgcgagaacgccaaagccaagacagaccacggggcggagatcgtgtacaagtcgccagtggtgtctggggacacgtctccacggcatctcagcaatgtctcctccaccggcagcatcgacatggtagactcgccccagctcgccacgctagctgacgaggtgtctgcctccctggccaagcagggtttg

SEQ ID NO: 44 - protein, 412 aa, Homo sapiens
  SITE 300: note = misc_feature - The 'X' at location 300 stands for Lys, Asn, Arg, Ser, Thr, Ile, Met, Glu, Asp, Gly, Ala, Val, Gln, His, Pro, Leu, Tyr, Trp, Cys, or Phe.
  SITE 301: note = misc_feature - The 'X' at location 301 stands for Lys, Asn, Arg, Ser, Thr, Ile, Met, Glu, Asp, Gly, Ala, Val, Gln, His, Pro, Leu, Tyr, Trp, Cys, or Phe.
  SITE 302: note = misc_feature - The 'X' at location 302 stands for Lys, Asn, Arg, Ser, Thr, Ile, Met, Glu, Asp, Gly, Ala, Val, Gln, His, Pro, Leu, Tyr, Trp, Cys, or Phe.
MAEPRQEFEVMEDHAGTYGLGDRKDQGGYTMHQDQEGDTDAGLKESPLQTPTEDGSEEPGSETSDAKSTPTAEAEEAGIGDTPSLEDEAAGHVTQARMVSKSKDGTGSDDKKAKGADGKTKIATPRGAAPPGQKGQANATRIPAKTPPAPKTPPSSGEPPKSGDRSGYSSPGSPGTPGSRSRTPSLPTPPTREPKKVAVVRTPPKSPSSAKSRLQTAPVPMPDLKNVKSKIGSTENLKHQPGGGKVQIINKKLDLSNVQSKCGSKDNIKHVPGGGSVQIVYKPVDLSKVTSKCGSLGNIXXXPGGGQVEVKSEKLDFKDRVQSKIGSLDNITHVPGGGNKKIETHKLTFRENAKAKTDHGAEIVYKSPVVSGDTSPRHLSNVSSTGSIDMVDSPQLATLADEVSASLAKQGL

SEQ ID NO: 45 - DNA, 1323 bp, Homo sapiens
  source 1..1323: mol_type = other DNA
  misc_feature 985..993: note = n is a, c, g, or t
  CDS 1..1323
atggctgagccccgccaggagttcgaagtgatggaagatcacgctgggacgtacgggttgggggacaggaaagatcaggggggctacaccatgcaccaagaccaagagggtgacacggacgctggcctgaaagaatctcccctgcagacccccactgaggacggatctgaggaaccgggctctgaaacctctgatgctaagagcactccaacagcggaagatgtgacagcacccttagtggatgagggagctcccggcaagcaggctgccgcgcagccccacacggagatcccagaaggaaccacagctgaagaagcaggcattggagacacccccagcctggaagacgaagctgctggtcacgtgacccaagctcgcatggtcagtaaaagcaaagacgggactggaagcgatgacaaaaaagccaagggggctgatggtaaaacgaagatcgccacaccgcggggagcagcccctccaggccagaagggccaggccaacgccaccaggattccagcaaaaaccccgcccgctccaaagacaccacccagctctggtgaacctccaaaatcaggggatcgcagcggctacagcagccccggctccccaggcactcccggcagccgctcccgcaccccgtcccttccaaccccacccacccgggagcccaagaaggtggcagtggtccgtactccacccaagtcgccgtcttccgccaagagccgcctgcagacagcccccgtgcccatgccagacctgaagaatgtcaagtccaagatcggctccactgagaacctgaagcaccagccgggaggcgggaaggtgcagataattaataagaagctggatcttagcaacgtccagtccaagtgtggctcaaaggataatatcaaacacgtcccgggaggcggcagtgtgcaaatagtctacaaaccagttgacctgagcaaggtgacctccaagtgtggctcattaggcaacatcnnnnnnnnnccaggaggtggccaggtggaagtaaaatctgagaagcttgacttcaaggacagagtccagtcgaagattgggtccctggacaatatcacccacgtccctggcggaggaaataaaaagattgaaacccacaagctgaccttccgcgagaacgccaaagccaagacagaccacggggcggagatcgtgtacaagtcgccagtggtgtctggggacacgtctccacggcatctcagcaatgtctcctccaccggcagcatcgacatggtagactcgccccagctcgccacgctagctgacgaggtgtctgcctccctggccaagcagggtttg

SEQ ID NO: 46 - protein, 441 aa, Homo sapiens
  SITE 329: note = misc_feature - The 'X' at location 329 stands for Lys, Asn, Arg, Ser, Thr, Ile, Met, Glu, Asp, Gly, Ala, Val, Gln, His, Pro, Leu, Tyr, Trp, Cys, or Phe.
  SITE 330: note = misc_feature - The 'X' at location 330 stands for Lys, Asn, Arg, Ser, Thr, Ile, Met, Glu, Asp, Gly, Ala, Val, Gln, His, Pro, Leu, Tyr, Trp, Cys, or Phe.
  SITE 331: note = misc_feature - The 'X' at location 331 stands for Lys, Asn, Arg, Ser, Thr, Ile, Met, Glu, Asp, Gly, Ala, Val, Gln, His, Pro, Leu, Tyr, Trp, Cys, or Phe.
MAEPRQEFEVMEDHAGTYGLGDRKDQGGYTMHQDQEGDTDAGLKESPLQTPTEDGSEEPGSETSDAKSTPTAEDVTAPLVDEGAPGKQAAAQPHTEIPEGTTAEEAGIGDTPSLEDEAAGHVTQARMVSKSKDGTGSDDKKAKGADGKTKIATPRGAAPPGQKGQANATRIPAKTPPAPKTPPSSGEPPKSGDRSGYSSPGSPGTPGSRSRTPSLPTPPTREPKKVAVVRTPPKSPSSAKSRLQTAPVPMPDLKNVKSKIGSTENLKHQPGGGKVQIINKKLDLSNVQSKCGSKDNIKHVPGGGSVQIVYKPVDLSKVTSKCGSLGNIXXXPGGGQVEVKSEKLDFKDRVQSKIGSLDNITHVPGGGNKKIETHKLTFRENAKAKTDHGAEIVYKSPVVSGDTSPRHLSNVSSTGSIDMVDSPQLATLADEVSASLAKQGL

SEQ ID NO: 47 - DNA, 126 bp, Homo sapiens; identical to SEQ ID NO: 31
  source 1..126: mol_type = other DNA
  misc_feature 82..84: note = n is a, c, g, or t, or deletion.
  misc_feature 100..102: note = n is a, c, g, or t, or deletion.
  misc_feature 106..108: note = n is a, c, g, or t, or deletion.
  CDS 1..126

SEQ ID NO: 48 - protein, 42 aa, Homo sapiens; identical to SEQ ID NO: 32
  SITE 28: note = misc_feature - The 'X' at location 28 stands for Lys, Asn, Arg, Ser, Thr, Ile, Met, Glu, Asp, Gly, Ala, Val, Gln, His, Pro, Leu, Tyr, Trp, Cys, or Phe.
  SITE 34: note = misc_feature - The 'X' at location 34 stands for Lys, Asn, Arg, Ser, Thr, Ile, Met, Glu, Asp, Gly, Ala, Val, Gln, His, Pro, Leu, Tyr, Trp, Cys, or Phe.
  SITE 36: note = misc_feature - The 'X' at location 36 stands for Lys, Asn, Arg, Ser, Thr, Ile, Met, Glu, Asp, Gly, Ala, Val, Gln, His, Pro, Leu, Tyr, Trp, Cys, or Phe.

SEQ ID NO: 49 - DNA, 43 bp, synthetic construct
  misc_feature 1..43: note = Synthetic DNA
  source 1..43: mol_type = other DNA
gtgttctctatgtaggctccgcaaccaaggagggagtggtgca

SEQ ID NO: 50 - DNA, 43 bp, synthetic construct
  misc_feature 1..43: note = Synthetic DNA
  source 1..43: mol_type = other DNA
tgcaccactccctccttggttgcggagcctacatagagaacac

SEQ ID NO: 51 - DNA, 43 bp, synthetic construct
  misc_feature 1..43: note = Synthetic DNA
  source 1..43: mol_type = other DNA
tctatgtaggctccaaaaccgcggagggagtggtgcatggtgt

SEQ ID NO: 52 - DNA, 43 bp, synthetic construct
  misc_feature 1..43: note = Synthetic DNA
  source 1..43: mol_type = other DNA
acaccatgcaccactccctccgcggttttggagcctacataga

SEQ ID NO: 53 - DNA, 43 bp, synthetic construct
  misc_feature 1..43: note = Synthetic DNA
  source 1..43: mol_type = other DNA
gtgttctctatgtaggctccagaaccaaggagggagtggtgca

SEQ ID NO: 54 - DNA, 43 bp, synthetic construct
  misc_feature 1..43: note = Synthetic DNA
  source 1..43: mol_type = other DNA
tgcaccactccctccttggttctggagcctacatagagaacac

SEQ ID NO: 55 - DNA, 43 bp, synthetic construct
  misc_feature 1..43: note = Synthetic DNA
  source 1..43: mol_type = other DNA
tctatgtaggctccaaaaccagggagggagtggtgcatggtgt

SEQ ID NO: 56 - DNA, 43 bp, synthetic construct
  misc_feature 1..43: note = Synthetic DNA
  source 1..43: mol_type = other DNA
acaccatgcaccactccctccctggttttggagcctacataga

SEQ ID NO: 57 - DNA, 57 bp, synthetic construct
  misc_feature 1..57: note = Synthetic DNA
  source 1..57: mol_type = other DNA
gagggtgttctctatgtaggctccgcaaccgcggagggagtggtgcatggtgtggca

SEQ ID NO: 58 - DNA, 57 bp, synthetic construct
  misc_feature 1..57: note = Synthetic DNA
  source 1..57: mol_type = other DNA
tgccacaccatgcaccactccctccgcggttgcggagcctacatagagaacaccctc

SEQ ID NO: 59 - DNA, 57 bp, synthetic construct
  misc_feature 1..57: note = Synthetic DNA
  source 1..57: mol_type = other DNA
gagggtgttctctatgtaggctcccgaacccgggagggagtggtgcatggtgtggca

SEQ ID NO: 60 - DNA, 57 bp, synthetic construct
  misc_feature 1..57: note = Synthetic DNA
  source 1..57: mol_type = other DNA
tgccacaccatgcaccactccctcccgggttcgggagcctacatagagaacaccctc

SEQ ID NO: 61 - DNA, 51 bp, synthetic construct
  misc_feature 1..51: note = Synthetic DNA
  source 1..51: mol_type = other DNA
tccaaaaccaaggagggagtggtggctggtgtggcaacagtggctgagaag

SEQ ID NO: 62 - DNA, 51 bp, synthetic construct
  misc_feature 1..51: note = Synthetic DNA
  source 1..51: mol_type = other DNA
cttctcagccactgttgccacaccagccaccactccctccttggttttgga

SEQ ID NO: 63 - DNA, 57 bp, synthetic construct
  misc_feature 1..57: note = Synthetic DNA
  source 1..57: mol_type = other DNA
gagggtgttctctatgtaggctccgaaaccgaggagggagtggtgcatggtgtggca

SEQ ID NO: 64 - DNA, 57 bp, synthetic construct
  misc_feature 1..57: note = Synthetic DNA
  source 1..57: mol_type = other DNA
tgccacaccatgcaccactccctcctcggtttcggagcctacatagagaacaccctc

SEQ ID NO: 65 - DNA, 29 bp, synthetic construct
  misc_feature 1..29: note = Synthetic DNA
  source 1..29: mol_type = other DNA
accgagggagtggtgcatggtgtggcaac

SEQ ID NO: 66 - DNA, 30 bp, synthetic construct
  misc_feature 1..30: note = Synthetic DNA
  source 1..30: mol_type = other DNA
ggagcctacatagagaacaccctcttttgt

SEQ ID NO: 67 - DNA, 25 bp, synthetic construct
  source 1..25: mol_type = other DNA
gtggaagtaaaatctgagaagcttg

SEQ ID NO: 68 - DNA, 25 bp, synthetic construct
  source 1..25: mol_type = other DNA
atgatggatgttgcctaatgagcca

SEQ ID NO: 69 - DNA, 25 bp, synthetic construct
  source 1..25: mol_type = other DNA
caggtggaagtaaaatctgagaagc

SEQ ID NO: 70 - DNA, 25 bp, synthetic construct
  source 1..25: mol_type = other DNA
tttatgatggatgttgcctaatgag